European Patent Application EP 4 335 871 A1, published March 13, 2024. Title: Tie2 Agonistic Antibodies and Uses Thereof. Applicant: Institute for Basic Science korea advanced institute of science and technology. The sequence listing filed with the application follows.

SEQUENCE LISTING (36 sequences)

SEQ ID NO: 1 - protein, 115 aa, Artificial Sequence
  hTAAB VH
QVQLQQPGAELVRPGASVKLSCKASGYSFTSYWMNWVKQRPGQGLEWIGMIHPSDSETRLNQKFMDKATLTVDKSSSTAYMQLSSPTSEDSAVYYCARGLYGNSWGQGTLVTVSA

SEQ ID NO: 2 - protein, 107 aa, Artificial Sequence
  hTAAB VL
DIQMTQSPSSLSASLGERVSLTCRASQDIGISLNWLQQEPDGTIKRLIYATSSLDSGVPKRFSGSRSGSDYSLTISSLESEDFVDYYCLQYASSPYTFGGGTKLEIK

SEQ ID NO: 3 - protein, 103 aa, Artificial Sequence
  hTAAB heavy chain constant region
AKTTPPSVYPLAPGSAAQTNSMVTLGCLVKGYFPEPVTVTWNSGSLSSGVHTFPAVLQSDLYTLSSSVTVPSSPRPSETVTCNVAHPASSTKVDKKIVPRDCG

SEQ ID NO: 4 - protein, 107 aa, Artificial Sequence
  hTAAB light chain constant region
RADAAPTVSIFPPSSEQLTSGGASVVCFLNNFYPKDINVKWKIDGSERQNGVLNSWTDQDSKDSTYSMSSTLTLTKDEYERHNSYTCEATHKTSTSPIVKSFNRNEC

SEQ ID NO: 5 - protein, 115 aa, Artificial Sequence
  hzTAAB-H1L1 VH
QVQLVQSGAEVKKPGASVKVSCKASGYSFTSYWMHWVRQAPGQGLEWMGIIHPSDSETRYAQKFQGRVTMTRDTSTSTVYMELSSLRSEDTAVYYCARGLYGNSWGQGTLVTVSS

SEQ ID NO: 6 - protein, 107 aa, Artificial Sequence
  hzTAAB-H1L1 VL
DIQMTQSPSSLSASVGDRVTITCRASQDIGISLGWYQQKPGKAPKRLIYATSSLQSGVPSRFSGSGSGTEFTLTISSLQPEDFATYYCLQYASSPYTFGQGTKLEIK

SEQ ID NO: 7 - protein, 115 aa, Artificial Sequence
  hzTAAB-H2L1 VH
QVQLVQSGAEVKKPGASVKVSCKASGYSFTSYWMHWVRQAPGQGLEWMGIIHPSDSETRYAQKFQGRVTMTVDKSTSTVYMELSSLRSEDTAVYYCARGLYGNSWGQGTLVTVSS

SEQ ID NO: 8 - protein, 107 aa, Artificial Sequence
  hzTAAB-H1L2 VL
DIQMTQSPSSLSASVGDRVTITCRASQDIGISLNWLQQKPGKAPKRLIYATSSLDSGVPSRFSGSRSGTEFTLTISSLQPEDFATYYCLQYASSPYTFGQGTKLEIK

SEQ ID NO: 9 - DNA, 345 bp, Artificial Sequence
  hTAAB VH
caggtccaactgcagcagcctggggctgagctggtgaggcctggagcttcagtgaagctgtcctgcaaggcttctggctactccttcaccagctactggatgaactgggtgaagcagaggcctggacaaggccttgagtggattggcatgattcatccttccgatagtgaaactaggttaaatcagaagttcatggacaaggccacattgactgtagacaaatcctccagcacagcctacatgcagctcagcagcccgacatctgaggactctgcggtctattactgtgctcgtggcctctatggtaactcttggggccaagggactctggtcactgtctctgca

SEQ ID NO: 10 - DNA, 321 bp, Artificial Sequence
  hTAAB VL
gacatccagatgacccagtctccatcctccttatctgcctctctgggagaaagagtcagtctcacttgtcgggcaagtcaggacattggtattagcttaaactggcttcagcaggaaccagatggaactattaaacgcctgatctacgccacatccagtttagattctggtgtccccaaaaggttcagtggcagtaggtctgggtcagattattctctcaccatcagcagccttgagtctgaagattttgtagactattactgtctacaatatgctagttctccgtacacgttcggaggggggaccaagctggaaataaaa

SEQ ID NO: 11 - DNA, 345 bp, Artificial Sequence
  hzTAAB-H1L1 VH
caggttcagctggtccagagcggggctgaggtcaagaaaccaggtgcatccgttaaggtgtcatgtaaagcctcggggtacagtttcaccagctactggatgcactgggtgagacaggcccctggtcaaggccttgaatggatgggaattatccatccctccgattccgaaactagatatgcacaaaagtttcagggcagagtgactatgaccagagacacatctacgtctaccgtctatatggagttgtcaagtctgcgcagcgaggacacagctgtatactattgcgccaggggactctatggcaatagctggggacagggcactctggtgacagtgtcttca

SEQ ID NO: 12 - DNA, 321 bp, Artificial Sequence
  hzTAAB-H1L1 VL
gatatccagatgactcaatctcctagctccctcagcgcttcagtgggcgacagagtcaccattacctgtcgcgcttctcaggatatcgggattagcctgggatggtaccagcagaagcctggtaaggcacccaaacggctgatttacgccacatcgagtctgcagtctggagtgccaagcaggttttcaggaagcgggtccggcaccgagtttactctgacaatatctagtctgcagccagaagacttcgccacatactattgcttgcagtatgcatcctcaccctatacgttcggccaaggaaccaaacttgagatcaag

SEQ ID NO: 13 - DNA, 345 bp, Artificial Sequence
  hzTAAB-H2L1 VH
caggtccagctggtgcagagtggcgccgaggtcaagaagcctggagcatcagttaaagtgtcttgtaaagctagtggctactcgtttacttcttactggatgcactgggtgagacaagccccaggtcaaggattggagtggatgggcattatccatcccagcgactccgaaacgagatatgctcagaagttccaggggcgggtgacaatgaccgtcgataaatctacaagcaccgtgtacatggagctttccagtctgagatccgaagacactgccgtatactattgcgcaaggggcctctatggtaattcatggggacaggggaccctggtgacagttagctcc

SEQ ID NO: 14 - DNA, 321 bp, Artificial Sequence
  hzTAAB-H1L2 VL
gacatccaaatgactcagagcccctccagtctgtcggcatctgtgggagatcgcgtcaccattacatgccgggccagccaggacatcggcattagtttgaactggcttcagcagaagcctgggaaagccccaaaaagactcatatacgctacttcttccctcgactctggcgtgccctcaagatttagcggaagcaggtcaggcactgagttcaccctgacaattagctccctgcaaccagaagatttcgctacatactattgtctgcagtacgcctcatccccttatacctttggtcaggggactaagctggagatcaag

SEQ ID NO: 15 - protein, 115 aa, Artificial Sequence
  3H7H12G4 VH
QVQLVQSGAEVKKPGASVKVSCKASGYTFTSYWMNWVRQAPGQGLEWMGMIHPSDSETRLNQKFMDRVTMTRDTSTSTVYMELSSLRSEDTAVYYCARGLYGNSWGQGTLVTVSS

SEQ ID NO: 16 - protein, 107 aa, Artificial Sequence
  3H7H12G4 VL
DIQMTQSPSSLSASVGDRVTITCRASQDIGISLNWLQQEPGKAPKRLIYATSSLDSGVPKRFSGSGSGTEFTLTISSLQPEDFATYYCLQYASSPYTFGQGTKVEIK

SEQ ID NO: 17 - DNA, 345 bp, Artificial Sequence
  3H7H12G4 VH
caggtgcagctggtccaatccggggctgaggtgaagaagcctggagcatcagtgaaagtttcatgcaaagctagtggttacaccttcaccagctattggatgaactgggtgcggcaggcccccggtcaggggcttgagtggatgggcatgatccacccatccgactctgagactaggctgaaccagaagtttatggatagagtgaccatgacaagagatacgtccacttctactgtctatatggaactgagcagtctgagatctgaagacacagccgtttactactgtgctcgcggactctatggcaatagctggggccaaggaacattggtaaccgtctcttct

SEQ ID NO: 18 - DNA, 321 bp, Artificial Sequence
  3H7H12G4 VL
gacatccagatgactcagtccccctcgagcctctcagcttctgttggagacagagtgacaattacatgccgggcctcacaggatattgggatctccctgaactggctgcaacaggaaccaggaaaggcccctaagcgcctgatatatgccacatcctctcttgactcaggggtcccaaagaggtttagcggcagtggatcaggtactgagttcactctcaccatctctagcctgcagcctgaggattttgcaacctactattgtttgcaatacgctagttccccctacacgttcggccagggcaccaaagtggaaatcaaa

SEQ ID NO: 19 - protein, 390 aa, Artificial Sequence
  Human Tie2 Ig3-Fn3 349T-738P
TPKIVDLPDHIEVNSGKFNPICKASGWPLPTNEEMTLVKPDGTVLHPKDFNHTDHFSVAIFTIHRILPPDSGVWVCSVNTVAGMVEKPFNISVKVLPKPLNAPNVIDTGHNFAVINISSEPYFGDGPIKSKKLLYKPVNHYEAWQHIQVTNEIVTLNYLEPRTEYELCVQLVRRGEGGEGHPGPVRRFTTASIGLPPPRGLNLLPKSQTTLNLTWQPIFPSSEDDFYVEVERRSVQKSDQQNIKVPGNLTSVLLNNLHPREQYVVRARVNTKAQGEWSEDLTAWTLSDILPPQPENIKISNITHSSAVISWTILDGYSISSITIRYKVQGKNEDQHVDVKIKNATITQYQLKGLEPETAYQVDIFAENNIGSSNPAFSHELVTLPESQAP

SEQ ID NO: 20 - DNA, 1170 bp, Artificial Sequence
  Human Tie2 Ig3-Fn3 349T-738P
accccaaagatagtggatttgccagatcatatagaagtaaacagtggtaaatttaatcccatttgcaaagcttctggctggccgctacctactaatgaagaaatgaccctggtgaagccggatgggacagtgctccatccaaaagactttaaccatacggatcatttctcagtagccatattcaccatccaccggatcctcccccctgactcaggagtttgggtctgcagtgtgaacacagtggctgggatggtggaaaagcccttcaacatttctgttaaagttcttccaaagcccctgaatgccccaaacgtgattgacactggacataactttgctgtcatcaacatcagctctgagccttactttggggatggaccaatcaaatccaagaagcttctatacaaacccgttaatcactatgaggcttggcaacatattcaagtgacaaatgagattgttacactcaactatttggaacctcggacagaatatgaactctgtgtgcaactggtccgtcgtggagagggtggggaagggcatcctggacctgtgagacgcttcacaacagcttctatcggactccctcctccaagaggtctaaatctcctgcctaaaagtcagaccactctaaatttgacctggcaaccaatatttccaagctcggaagatgacttttatgttgaagtggagagaaggtctgtgcaaaaaagtgatcagcagaatattaaagttccaggcaacttgacttcggtgctacttaacaacttacatcccagggagcagtacgtggtccgagctagagtcaacaccaaggcccagggggaatggagtgaagatctcactgcttggacccttagtgacattcttcctcctcaaccagaaaacatcaagatttccaacattacacactcctcggctgtgatttcttggacaatattggatggctattctatttcttctattactatccgttacaaggttcaaggcaagaatgaagaccagcacgttgatgtgaagataaagaatgccaccatcactcagtatcagctcaagggcctagagcctgaaacagcataccaggtggacatttttgcagagaacaacatagggtcaagcaacccagccttttctcatgaactggtgaccctcccagaatctcaagcacca

SEQ ID NO: 21 - protein, 195 aa, Artificial Sequence
  Human Tie2 Fn2-3 541I-735S
IGLPPPRGLNLLPKSQTTLNLTWQPIFPSSEDDFYVEVERRSVQKSDQQNIKVPGNLTSVLLNNLHPREQYVVRARVNTKAQGEWSEDLTAWTLSDILPPQPENIKISNITHSSAVISWTILDGYSISSITIRYKVQGKNEDQHVDVKIKNATITQYQLKGLEPETAYQVDIFAENNIGSSNPAFSHELVTLPES

SEQ ID NO: 22 - DNA, 585 bp, Artificial Sequence
  Human Tie2 Fn2-3 541I-735S
atcggactccctcctccaagaggtctaaatctcctgcctaaaagtcagaccactctaaatttgacctggcaaccaatatttccaagctcggaagatgacttttatgttgaagtggagagaaggtctgtgcaaaaaagtgatcagcagaatattaaagttccaggcaacttgacttcggtgctacttaacaacttacatcccagggagcagtacgtggtccgagctagagtcaacaccaaggcccagggggaatggagtgaagatctcactgcttggacccttagtgacattcttcctcctcaaccagaaaacatcaagatttccaacattacacactcctcggctgtgatttcttggacaatattggatggctattctatttcttctattactatccgttacaaggttcaaggcaagaatgaagaccagcacgttgatgtgaagataaagaatgccaccatcactcagtatcagctcaagggcctagagcctgaaacagcataccaggtggacatttttgcagagaacaacatagggtcaagcaacccagccttttctcatgaactggtgaccctcccagaatct

SEQ ID NO: 23 - protein, 330 aa, Artificial Sequence
  Human IgG1 heavy chain constant region
ASTKGPSVFPLAPSSKSTSGGTAALGCLVKDYFPEPVTVSWNSGALTSGVHTFPAVLQSSGLYSLSSVVTVPSSSLGTQTYICNVNHKPSNTKVDKKVEPKSCDKTHTCPPCPAPELLGGPSVFLFPPKPKDTLMISRTPEVTCVVVDVSHEDPEVKFNWYVDGVEVHNAKTKPREEQYNSTYRVVSVLTVLHQDWLNGKEYKCKVSNKALPAPIEKTISKAKGQPREPQVYTLPPSREEMTKNQVSLTCLVKGFYPSDIAVEWESNGQPENNYKTTPPVLDSDGSFFLYSKLTVDKSRWQQGNVFSCSVMHEALHNHYTQKSLSLSPGK

SEQ ID NO: 24 - DNA, 990 bp, Artificial Sequence
  Human IgG1 heavy chain constant region
gctagcaccaagggcccatcggtcttccccctggcaccctcctccaagagcacctctgggggcacagcggccctgggctgcctggtcaaggactacttccccgaaccggtgacggtgtcgtggaactcaggcgccctgaccagcggcgtgcacaccttcccggctgtcctacagtcctcaggactctactccctcagcagcgtggtgaccgtgccctccagcagcttgggcacccagacctacatctgcaacgtgaatcacaagcccagcaacaccaaggtggacaagaaagttgagcccaaatcttgtgacaaaactcacacatgcccaccgtgcccagcacctgaactcctggggggaccgtcagtcttcctcttccccccaaaacccaaggacaccctcatgatctcccggacccctgaggtcacatgcgtggtggtggacgtgagccacgaagaccctgaggtcaagttcaactggtacgtggacggcgtggaggtgcataatgccaagacaaagccgcgggaggagcagtacaacagcacgtaccgtgtggtcagcgtcctcaccgtcctgcaccaggactggctgaatggcaaggagtacaagtgcaaggtctccaacaaagccctcccagcccccatcgagaaaaccatctccaaagccaaagggcagccccgagaaccacaggtgtacaccctgcccccatcccgggaggagatgaccaagaaccaggtcagcctgacctgcctggtcaaaggcttctatcccagcgacatcgccgtggagtgggagagcaatgggcagccggagaacaactacaagaccacgcctcccgtgctggactccgacggctccttcttcctctacagcaagctcaccgtggacaagagcaggtggcagcaggggaacgtcttctcatgctccgtgatgcatgaggctctgcacaaccactacacgcagaagagcctctccctgtctccgggtaaa

SEQ ID NO: 25 - protein, 326 aa, Artificial Sequence
  Human IgG2 heavy chain constant region
ASTKGPSVFPLAPCSRSTSESTAALGCLVKDYFPEPVTVSWNSGALTSGVHTFPAVLQSSGLYSLSSVVTVPSSNFGTQTYTCNVDHKPSNTKVDKTVERKCCVECPPCPAPPVAGPSVFLFPPKPKDTLMISRTPEVTCVVVDVSHEDPEVQFNWYVDGVEVHNAKTKPREEQFNSTFRVVSVLTVVHQDWLNGKEYKCKVSNKGLPAPIEKTISKTKGQPREPQVYTLPPSREEMTKNQVSLTCLVKGFYPSDIAVEWESNGQPENNYKTTPPMLDSDGSFFLYSKLTVDKSRWQQGNVFSCSVMHEALHNHYTQKSLSLSPGK

SEQ ID NO: 26 - DNA, 978 bp, Artificial Sequence
  Human IgG2 heavy chain constant region
gctagcaccaagggcccatcggtcttccccctggcgccctgctccaggagcacctccgagagcacagcggccctgggctgcctggtcaaggactacttccccgaaccggtgacggtgtcgtggaactcaggcgctctgaccagcggcgtgcacaccttcccagctgtcctacagtcctcaggactctactccctcagcagcgtggtgaccgtgccctccagcaacttcggcacccagacctacacctgcaacgtagatcacaagcccagcaacaccaaggtggacaagacagttgagcgcaaatgttgtgtcgagtgcccaccgtgcccagcaccacctgtggcaggaccgtcagtcttcctcttccccccaaaacccaaggacaccctcatgatctcccggacccctgaggtcacgtgcgtggtggtggacgtgagccacgaagaccccgaggtccagttcaactggtacgtggacggcgtggaggtgcataatgccaagacaaagccacgggaggagcagttcaacagcacgttccgtgtggtcagcgtcctcaccgttgtgcaccaggactggctgaacggcaaggagtacaagtgcaaggtctccaacaaaggcctcccagcccccatcgagaaaaccatctccaaaaccaaagggcagccccgagaaccacaggtgtacaccctgcccccatcccgggaggagatgaccaagaaccaggtcagcctgacctgcctggtcaaaggcttctaccccagcgacatcgccgtggagtgggagagcaatgggcagccggagaacaactacaagaccacgcctcccatgctggactccgacggctccttcttcctctacagcaagctcaccgtggacaagagcaggtggcagcaggggaacgtcttctcatgctccgtgatgcatgaggctctgcacaaccactacacgcagaagagcctctccctgtctccgggtaaa

SEQ ID NO: 27 - protein, 327 aa, Artificial Sequence
  Human IgG4 heavy chain constant region
ASTKGPSVFPLAPCSRSTSESTAALGCLVKDYFPEPVTVSWNSGALTSGVHTFPAVLQSSGLYSLSSVVTVPSSSLGTKTYTCNVDHKPSNTKVDKRVESKYGPPCPSCPAPEFLGGPSVFLFPPKPKDTLMISRTPEVTCVVVDVSQEDPEVQFNWYVDGVEVHNAKTKPREEQFNSTYRVVSVLTVLHQDWLNGKEYKCKVSNKGLPSSIEKTISKAKGQPREPQVYTLPPSQEEMTKNQVSLTCLVKGFYPSDIAVEWESNGQPENNYKTTPPVLDSDGSFFLYSRLTVDKSRWQEGNVFSCSVMHEALHNHYTQKSLSLSLGK

SEQ ID NO: 28 - DNA, 981 bp, Artificial Sequence
  Human IgG4 heavy chain constant region
gctagcaccaagggcccatcggtcttccccctggcgccctgctccaggagcacctccgagagcacagccgccctgggctgcctggtcaaggactacttccccgaaccggtgacggtgtcgtggaactcaggcgccctgaccagcggcgtgcacaccttcccggctgtcctacagtcctcaggactctactccctcagcagcgtggtgaccgtgccctccagcagcttgggcacgaagacctacacctgcaacgtagatcacaagcccagcaacaccaaggtggacaagagagttgagtccaaatatggtcccccatgcccatcatgcccagcacctgagttcctggggggaccatcagtcttcctgttccccccaaaacccaaggacactctcatgatctcccggacccctgaggtcacgtgcgtggtggtggacgtgagccaggaagaccccgaggtccagttcaactggtacgtggatggcgtggaggtgcataatgccaagacaaagccgcgggaggagcagttcaacagcacgtaccgtgtggtcagcgtcctcaccgtcctgcaccaggactggctgaacggcaaggagtacaagtgcaaggtctccaacaaaggcctcccgtcctccatcgagaaaaccatctccaaagccaaagggcagccccgagagccacaggtgtacaccctgcccccatcccaggaggagatgaccaagaaccaggtcagcctgacctgcctggtcaaaggcttctaccccagcgacatcgccgtggagtgggagagcaatgggcagccggagaacaactacaagaccacgcctcccgtgctggactccgacggctccttcttcctctacagcaggctcaccgtggacaagagcaggtggcaggaggggaatgtcttctcatgctccgtgatgcatgaggctctgcacaaccactacacacagaagagcctctccctgtctctgggtaaa

SEQ ID NO: 29 - protein, 106 aa, Artificial Sequence
  Human Kappa light chain constant region
TVAAPSVFIFPPSDEQLKSGTASVVCLLNNFYPREAKVQWKVDNALQSGNSQESVTEQDSKDSTYSLSSTLTLSKADYEKHKVYACEVTHQGLSSPVTKSFNRGEC

SEQ ID NO: 30 - DNA, 318 bp, Artificial Sequence
  Human Kappa light chain constant region
acggtggctgcaccatctgtcttcatcttcccgccatctgatgagcagttgaaatctggaactgcctctgttgtgtgcctgctgaataacttctatcccagagaggccaaagtacagtggaaggtggataacgccctccaatcgggtaactcccaggagagtgtcacagagcaggacagcaaggacagcacctacagcctcagcagcaccctgacgctgagcaaagcagactacgagaaacacaaagtctacgcctgcgaagtcacccatcagggcctgagctcgcccgtcacaaagagcttcaacaggggagagtgc

SEQ ID NO: 31 - protein, 106 aa, Artificial Sequence; identical to SEQ ID NO: 29
  Human Kappa light chain constant region

SEQ ID NO: 32 - DNA, 318 bp, Artificial Sequence; identical to SEQ ID NO: 30
  Human Kappa light chain constant region

SEQ ID NO: 33 - protein, 330 aa, Artificial Sequence; identical to SEQ ID NO: 23
  Human IgG1 heavy chain constant region

SEQ ID NO: 34 - DNA, 990 bp, Artificial Sequence; identical to SEQ ID NO: 24
  Human IgG1 heavy chain constant region

SEQ ID NO: 35 - protein, 309 aa, Artificial Sequence
  hTAAB heavy chain constant region
GCTAAAACCACACCTCCCAGCGTGTACCCTCTGGCCCCAGGATCAGCAGCCCAGACCAATAGCATGGTGACACTCGGATGCCTGGTAAAGGGCTATTTCCCTGAGCCTGTGACGGTCACTTGGAATAGTGGGAGTTTGTCTAGTGGTGTTCACACATTTCCCGCTGTCCTGCAGAGCGATTTATACACACTTAGCTCCTCTGTGACCGTGCCATCCTCTCCTAGACCGTCAGAAACTGTGACTTGTAACGTCGCCCATCCAGCATCATCCACCAAAGTTGACAAGAAGATCGTTCCCAGAGACTGTGGC

SEQ ID NO: 36 - DNA, 321 bp, Artificial Sequence
  hTAAB light chain constant region
cgcgctgatgccgctcctaccgtctccatatttccgccctcctcagagcagctcacatcaggtggggcgtccgtggtgtgctttctgaataatttctatccgaaggatattaacgtcaaatggaaaattgacggctcggaacgtcaaaacggtgttctgaactcctggaccgaccaggattctaaggatagtacttatagtatgagtagcacattgacacttactaaagacgaatatgagcgtcacaatagctacacctgtgaggccacccataaaacgagcacctcgccgatcgttaagagctttaatcgcaatgaatgc